European Patent Specification EP 4 301 868 B1, published May 6, 2026. Title: METHODS AND COMPOSITIONS FOR COMBINATORIAL TARGETING OF THE CELL TRANSCRIPTOME. Applicant: New York Genome Center, Inc. New York University. The sequence listing filed with the application follows.

SEQUENCE LISTING (44 sequences)

SEQ ID NO: 1 - RNA, 88 nt, Artificial Sequence
  synthetic construct
  misc_feature (52)..(66): n is a, c, g, or u
aaccccuaccaacuggucgggguucaaaguccuuggcacccgagaauuccannnnnnnnnnnnnnngcuuuaaggccgguccuagcaa

SEQ ID NO: 2 - DNA, 22 bp, Artificial Sequence
  synthetic construct
ttgctaggaccggccttaaagc

SEQ ID NO: 3 - DNA, 72 bp, Artificial Sequence
  synthetic construct
  misc_feature (23)..(50): n is a, c, g, or t
gtcagatgtgtataagagacagnnnnnnnnnnnnnnnnnnnnnnnnnnnnttgctaggaccggccttaaagc

SEQ ID NO: 4 - RNA, 88 nt, Artificial Sequence
  synthetic construct
  misc_feature (52)..(66): n is a, c, g, or u
aaccccuaccaacuggucgggguuugaaacccuuggcacccgagaauuccannnnnnnnnnnnnnngcuuuaaggccgguccuagcaa

SEQ ID NO: 5 - DNA, 30 bp, Artificial Sequence
  synthetic constructs
aagcagtggtatcaacgcagagtacatggg

SEQ ID NO: 6 - DNA, 168 bp, Artificial Sequence
  synthetic construct
  misc_feature (23)..(50): n is a, c, g, or t
  misc_feature (73)..(87): n is a, c, g, or t
gtcagatgtgtataagagacagnnnnnnnnnnnnnnnnnnnnnnnnnnnnttgctaggaccggccttaaagcnnnnnnnnnnnnnnntggaattctcgggtgccaagggtttcaaaccccgaccagttggtaggggttcccatgtactctgcgttgataccactgctt

SEQ ID NO: 7 - DNA, 27 bp, Artificial Sequence
  synthetic construct
gcagcgtcagatgtgtataagagacag

SEQ ID NO: 8 - DNA, 22 bp, Artificial Sequence
  synthetic construct
aagcagtggtatcaacgcagag

SEQ ID NO: 9 - DNA, 173 bp, Artificial Sequence
  synthetic construct
  misc_feature (28)..(55): n is a, c, g, or t
  misc_feature (78)..(92): n is a, c, g, or t
gcagcgtcagatgtgtataagagacagnnnnnnnnnnnnnnnnnnnnnnnnnnnnttgctaggaccggccttaaagcnnnnnnnnnnnnnnntggaattctcgggtgccaagggtttcaaaccccgaccagttggtaggggttcccatgtactctgcgttgataccactgctt

SEQ ID NO: 10 - DNA, 173 bp, Artificial Sequence
  synthetic construct
  misc_feature (82)..(96): n is a, c, g, or t
  misc_feature (119)..(146): n is a, c, g, or t
aagcagtggtatcaacgcagagtacatgggaacccctaccaactggtcggggtttgaaacccttggcacccgagaattccannnnnnnnnnnnnnngctttaaggccggtcctagcaannnnnnnnnnnnnnnnnnnnnnnnnnnnctgtctcttatacacatctgacgctgc

SEQ ID NO: 11 - DNA, 27 bp, Artificial Sequence
  synthetic construct
gcagcgtcagatgtgtataagagacag

SEQ ID NO: 12 - DNA, 20 bp, Artificial Sequence
  synthetic construct
ccttggcacccgagaattcc

SEQ ID NO: 13 - DNA, 113 bp, Artificial Sequence
  synthetic construct
  misc_feature (28)..(55): n is a, c, g, or t
  misc_feature (78)..(92): n is a, c, g, or t
gcagcgtcagatgtgtataagagacagnnnnnnnnnnnnnnnnnnnnnnnnnnnnttgctaggaccggccttaaagcnnnnnnnnnnnnnnntggaattctcgggtgccaagg

SEQ ID NO: 14 - DNA, 113 bp, Artificial Sequence
  synthetic construct
  misc_feature (22)..(36): n is a, c, g, or t
  misc_feature (59)..(86): n is a, c, g, or t
ccttggcacccgagaattccannnnnnnnnnnnnnngctttaaggccggtcctagcaannnnnnnnnnnnnnnnnnnnnnnnnnnnctgtctcttatacacatctgacgctgc

SEQ ID NO: 15 - DNA, 62 bp, Artificial Sequence
  synthetic construct
aatgatacggcgaccaccgagatctacactcgtcggcagcgtcagatgtgtataagagacag

SEQ ID NO: 16 - DNA, 113 bp, Artificial Sequence; identical to SEQ ID NO: 13
  synthetic construct
  misc_feature (28)..(55): n is a, c, g, or t
  misc_feature (78)..(92): n is a, c, g, or t

SEQ ID NO: 17 - DNA, 113 bp, Artificial Sequence; identical to SEQ ID NO: 14
  synthetic construct
  misc_feature (22)..(36): n is a, c, g, or t
  misc_feature (59)..(86): n is a, c, g, or t

SEQ ID NO: 18 - DNA, 65 bp, Artificial Sequence
  synthetic construct
  misc_feature (25)..(32): n is a, c, g, or t
gttcgtcttctgccgtatgctctannnnnnnncactgacctcaaggaaccgtgggctcttaaggt

SEQ ID NO: 19 - DNA, 191 bp, Artificial Sequence
  synthetic construct
  misc_feature (62)..(89): n is a, c, g, or t
  misc_feature (112)..(126): n is a, c, g, or t
  misc_feature (160)..(167): n is a, c, g, or t
atgatacggcgaccaccgagatctacactcgtcggcagcgtcagatgtgtataagagacagnnnnnnnnnnnnnnnnnnnnnnnnnnnnttgctaggaccggccttaaagcnnnnnnnnnnnnnnntggaattctcgggtgccaaggaactccagtcacnnnnnnnnatctcgtatgccgtcttctgcttg

SEQ ID NO: 20 - DNA, 191 bp, Artificial Sequence
  synthetic construct
  misc_feature (25)..(32): n is a, c, g, or t
  misc_feature (66)..(80): n is a, c, g, or t
  misc_feature (103)..(130): n is a, c, g, or t
caagcagaagacggcatacgagatnnnnnnnngtgactggagttccttggcacccgagaattccannnnnnnnnnnnnnngctttaaggccggtcctagcaannnnnnnnnnnnnnnnnnnnnnnnnnnnctgtctcttatacacatctgacgctgccgacgagtgtagatctcggtggtcgccgtatcat

SEQ ID NO: 21 - RNA, 44 nt, Artificial Sequence
  synthetic construct
  misc_feature (8)..(22): n is a, c, g, or u
cgcagagnnnnnnnnnnnnnnngcuuuaaggccgguccuagcaa

SEQ ID NO: 22 - DNA, 22 bp, Artificial Sequence
  synthetic construct
ttgctaggaccggccttaaagc

SEQ ID NO: 23 - DNA, 16 bp, Artificial Sequence
  synthetic construct
baaaaaaaaaaaaaaa

SEQ ID NO: 24 - DNA, 16 bp, Artificial Sequence
  synthetic construct
tttttttttttttttv

SEQ ID NO: 25 - DNA, 23 bp, Artificial Sequence
  synthetic construct
gctaccgtcgctgtgttaacaga

SEQ ID NO: 26 - DNA, 23 bp, Artificial Sequence
  synthetic construct
tctgttaacacagcgacggtagc

SEQ ID NO: 27 - DNA, 24 bp, Artificial Sequence
  synthetic construct
tctgttaacaccggcgacggcctg

SEQ ID NO: 28 - DNA, 23 bp, Artificial Sequence
  synthetic construct
tctgttaacccagtgacagtagt

SEQ ID NO: 29 - DNA, 23 bp, Artificial Sequence
  synthetic construct
gaccgctcttcctgagtcactag

SEQ ID NO: 30 - DNA, 23 bp, Artificial Sequence
  synthetic construct
ctagtgactcaggaagagcggtc

SEQ ID NO: 31 - DNA, 24 bp, Artificial Sequence
  synthetic construct
agccggactcaaggaagagcggtc

SEQ ID NO: 32 - DNA, 24 bp, Artificial Sequence
  synthetic construct
ctagtgactcaaggagagagggtt

SEQ ID NO: 33 - DNA, 22 bp, Artificial Sequence
  synthetic construct
ctagtgacacaggaagacggaa

SEQ ID NO: 34 - DNA, 22 bp, Artificial Sequence
  synthetic construct
tgggtgacgcaggaaagcggtc

SEQ ID NO: 35 - DNA, 23 bp, Artificial Sequence
  synthetic construct
gataccctgataacgacactagc

SEQ ID NO: 36 - DNA, 23 bp, Artificial Sequence
  synthetic construct
gctagtgtcgttatcagggtatc

SEQ ID NO: 37 - DNA, 23 bp, Artificial Sequence
  synthetic construct
cctagtgtggttatcaaggtggt

SEQ ID NO: 38 - DNA, 23 bp, Artificial Sequence
  synthetic construct
gctagtgtcgatattagggtcgt

SEQ ID NO: 39 - RNA, 95 nt, Artificial Sequence
  synthetic construct
gaagguuucucucuuccugagaauacaacccguauuguauucucagguucugcucuuuggggccuuucccuagcuuaaaaaaaaaaagagcagaa

SEQ ID NO: 40 - RNA, 93 nt, Artificial Sequence
  synthetic construct
agguguuucucuuacugagugcagcccauggccgcacucagguucugcuuuacaccuucccaucugugaaagagugagcaggaaaaagcagaa

SEQ ID NO: 41 - RNA, 54 nt, Artificial Sequence
  synthetic construct
cuuggugcuuagcucuuucaccaaggauauuacacgcggaauaccgcaagggaa

SEQ ID NO: 42 - DNA, 55 bp, Artificial Sequence
  synthetic construct
cccaacggggggctgaaactcccaauaggacccaaguccccccccgaggacuggg

SEQ ID NO: 43 - DNA, 71 bp, Artificial Sequence
  synthetic construct
ugucaggccugcuagucagccacaguuuggggaaagcugugcagcctguaacccccccaggagaagcuggg

SEQ ID NO: 44 - RNA, 42 nt, Artificial Sequence
  synthetic construct
uugacgcgguucuaucuaguuacgcguuaaaccaacuagaaa